European Patent Application EP 4 814 004 A1, published September 30, 2026. Title: 一组阻断抗PD-1抗体与细胞表面PD-1分子结合的PD-1分子及其突变体和用途. Applicant: 河南省肿瘤医院. The sequence listing filed with the application follows.

SEQUENCE LISTING (5 sequences)

SEQ ID NO: 1 - protein, 170 aa, synthetic construct
MQIPQAPWPVVWAVLQLGWRPGWFLDSPDRPWNPPTFSPALLVVTEGDNATFTCSFSNTSESFVLNWYRMSPSNQTDKLAAFPEDRSQPGQDCRFRVTQLPNGRDFHMSVVRARRNDSGTYLCGAISLAPKAQIKESLRAELRVTERRAEVPTAHPSPSPRPAGQFQTLV

SEQ ID NO: 2 - protein, 170 aa, synthetic construct
MQIPQAPWPVVWAVLQLGWRPGWFLDSPDRPWNPPTFSPALLVVTEGDNATFTCSFSNTSESFVLNWYRMSPSNQTDKLAAFPEDRSQPGQDCRFRVTQLPNGRDFHMSVVRARRNDSGTYLCGAASLAPKAQIKESLRAELRVTERRAEVPTAHPSPSPRPAGQFQTLV

SEQ ID NO: 3 - protein, 170 aa, synthetic construct
MQIPQAPWPVVWAVLQLGWRPGWFLDSPDRPWNPPTFSPALLVVTEGDNATFTCSFSNTSESFVLNWYRMSPSNQTDKLAAFPEDRSQPGQDCRFRVTQLPNGRDFHMSVVRARRNDSGTYLCGAISLAPKAQAKESLRAELRVTERRAEVPTAHPSPSPRPAGQFQTLV

SEQ ID NO: 4 - DNA, 513 bp, synthetic construct
  source 1..513: mol_type = other DNA
atgcagatcccccaggctccttggcctgtggtgtgggctgtgctgcagctgggatggaggcctggatggttcctggactcccctgaccgtccttggaaccctcctaccttctcccccgctctcctcgttgtcaccgagggagataacgccaccttcacctgctccttctccaacacctccgagtccttcgtcctcaactggtatcgcatgtctccctccaaccaaaccgacaagctggccgctttccccgaagatagaagccaacccggccaggactgcagattccgtgtgacacagctgcccaacgggcgagatttccacatgagcgtcgtgagggccagaagaaacgactccgggacctacctgtgtggcgcagcttctctggctcccaaggctcaaatcaaagaaagcctccgggccgagctgagagtgactgaaagaagagctgaggtgcccaccgcccacccttctccttctcctagacccgctggacagttccaaaccctcgtgtga

SEQ ID NO: 5 - DNA, 513 bp, synthetic construct
  source 1..513: mol_type = other DNA
atgcagatcccccaggctccttggcctgtggtgtgggctgtgctgcagctgggatggaggcctggatggttcctggactcccctgaccgtccttggaaccctcctaccttctcccccgctctcctcgttgtcaccgagggagataacgccaccttcacctgctccttctccaacacctccgagtccttcgtcctcaactggtatcgcatgtctccctccaaccaaaccgacaagctggccgctttccccgaagatagaagccaacccggccaggactgcagattccgtgtgacacagctgcccaacgggcgagatttccacatgagcgtcgtgagggccagaagaaacgactccgggacctacctgtgtggcgcaatctccctggctccaaaagcccaagccaaagaaagcctccgggccgaactgagagtgaccgaaagaagagccgaggtgcccaccgcacacccttctccttcacctcgacctgctggacagttccaaaccctcgtgtga